European Patent Specification EP 3 313 866 B1, published November 20, 2024. Title: COMPOSITIONS AND METHODS FOR TREATING CANCER AND PROMOTING WOUND HEALING. Applicant: University of Louisville Research Foundation, Inc. Matoba, Nobuyuki Baldauf, Keegan Royal, Joshua. The sequence listing filed with the application follows.

SEQUENCE LISTING (31 sequences)

SEQ ID NO: 1 - DNA, 309 bp, Vibrio cholerae
accccacaaaacatcactgacttgtgtgctgagtaccacaacacccaaatccacaccctcaatgacaagatctttagctacaccgagagccttgctggcaagagggagatggctatcatcaccttcaagaatggtgctaccttccaagtggaggtgcctggaagccaacacattgatagccaaaagaaggccattgagaggatgaaggacacacttaggatagcttacctcactgaggctaaggtggagaagctttgtgtgtggaacaacaagaccccccatgctattgctgccatcagcatggccaac

SEQ ID NO: 2 - protein, 103 aa, Vibrio cholerae
TPQNITDLCAEYHNTQIHTLNDKIFSYTESLAGKREMAIITFKNGATFQVEVPGSQHIDSQKKAIERMKDTLRIAYLTEAKVEKLCVWNNKTPHAIAAISMAN

SEQ ID NO: 3 - DNA, 327 bp, Artificial Sequence
  Cholera Toxin B Subunit Polypeptide Variant Polypeptide
accccacaaagcatcactgacttgtgtgctgagtaccacaacacccaaatccacaccctcaatgacaagatctttagctacaccgagagccttgctggcaagagggagatggctatcatcaccttcaagaatggtgctaccttccaagtggaggtgcctggaagccaacacattgatagccaaaagaaggccattgagaggatgaaggacacacttaggatagcttacctcactgaggctaaggtggagaagctttgtgtgtggaacaacaagaccccccatgctattgctgccatcagcatggccaactccgagaaggatgaactc

SEQ ID NO: 4 - protein, 109 aa, Artificial Sequence
  Cholera Toxin B Subunit Polypeptide Variant Polypeptide
TPQSITDLCAEYHNTQIHTLNDKIFSYTESLAGKREMAIITFKNGATFQVEVPGSQHIDSQKKAIERMKDTLRIAYLTEAKVEKLCVWNNKTPHAIAAISMANSEKDEL

SEQ ID NO: 5 - DNA, 327 bp, Artificial Sequence
  Cholera Toxin B Subunit Polypeptide Variant Polypeptide
accccacaaaacatcactgacttgtgtgctgagtaccacaacacccaaatccacaccctcaatgacaagatctttagctacaccgagagccttgctggcaagagggagatggctatcatcaccttcaagaatggtgctaccttccaagtggaggtgcctggaagccaacacattgatagccaaaagaaggccattgagaggatgaaggacacacttaggatagcttacctcactgaggctaaggtggagaagctttgtgtgtggaacaacaagaccccccatgctattgctgccatcagcatggccaactccgagaaggatgaactc

SEQ ID NO: 6 - protein, 109 aa, Artificial Sequence
  Cholera Toxin B Subunit Polypeptide Variant Polypeptide
TPQNITDLCAEYHNTQIHTLNDKIFSYTESLAGKREMAIITFKNGATFQVEVPGSQHIDSQKKAIERMKDTLRIAYLTEAKVEKLCVWNNKTPHAIAAISMANSEKDEL

SEQ ID NO: 7 - DNA, 327 bp, Artificial Sequence
  Cholera Toxin B Subunit Polypeptide Variant Polypeptide
accccacaaaacatcactgacttgtgtgctgagtaccacaacacccaaatccacaccctcaatgacaagatctttagctacaccgagagccttgctggcaagagggagatggctatcatcaccttcaagaatggtgctaccttccaagtggaggtgcctggaagccaacacattgatagccaaaagaaggccattgagaggatgaaggacacacttaggatagcttacctcactgaggctaaggtggagaagctttgtgtgtggaacaacaagaccccccatgctattgctgccatcagcatggccaacgttactaaggatgaactc

SEQ ID NO: 8 - protein, 109 aa, Artificial Sequence
  Cholera Toxin B Subunit Polypeptide Variant Polypeptide
TPQNITDLCAEYHNTQIHTLNDKIFSYTESLAGKREMAIITFKNGATFQVEVPGSQHIDSQKKAIERMKDTLRIAYLTEAKVEKLCVWNNKTPHAIAAISMANVTKDEL

SEQ ID NO: 9 - DNA, 327 bp, Artificial Sequence
  Cholera Toxin B Subunit Polypeptide Variant Polypeptide
accccacaaaacatcactgacttgtgtgctgagtaccacaacacccaaatccacaccctcaatgacactatctttagctacaccgagagccttgctggcaagagggagatggctatcatcaccttcaagaatggtgctaccttccaagtggaggtgcctggaagccaacacattgatagccaaaagaaggccattgagaggatgaaggacacacttaggatagcttacctcactgaggctaaggtggagaagctttgtgtgtggaacaacaagaccccccatgctattgctgccatcagcatggccaactccgagaaggatgaactc

SEQ ID NO: 10 - protein, 109 aa, Artificial Sequence
  Cholera Toxin B Subunit Polypeptide Variant Polypeptide
TPQNITDLCAEYHNTQIHTLNDTIFSYTESLAGKREMAIITFKNGATFQVEVPGSQHIDSQKKAIERMKDTLRIAYLTEAKVEKLCVWNNKTPHAIAAISMANSEKDEL

SEQ ID NO: 11 - DNA, 327 bp, Artificial Sequence
  Cholera Toxin B Subunit Polypeptide Variant Polypeptide
accccacaaaacatcactgacttgtgtgctgagtaccacaacacccaaatccacaccctcaatgacactatctttagctacaccgagagccttgctggcaagagggagatggctatcatcaccttcaagaatggtgctaccttccaagtggaggtgcctggaagccaacacattgatagccaaaagaaggccattgagaggatgaaggacacacttaggatagcttacctcactgaggctaaggtggagaagctttgtgtgtggaacaacaagaccccccatgctattgctgccatcagcatggccaacgttactaaggatgaactc

SEQ ID NO: 12 - protein, 109 aa, Artificial Sequence
  Cholera Toxin B Subunit Polypeptide Variant Polypeptide
TPQNITDLCAEYHNTQIHTLNDTIFSYTESLAGKREMAIITFKNGATFQVEVPGSQHIDSQKKAIERMKDTLRIAYLTEAKVEKLCVWNNKTPHAIAAISMANVTKDEL

SEQ ID NO: 13 - DNA, 345 bp, Artificial Sequence
  Cholera Toxin B Subunit Polypeptide Variant Polypeptide
accccacaaaacatcactgacttgtgtgctgagtaccacaacacccaaatccacaccctcaatgacactatctttagctacaccgagagccttgctggcaagagggagatggctatcatcaccttcaagaatggtgctaccttccaagtggaggtgcctggaagccaacacattgatagccaaaagaaggccattgagaggatgaaggacacacttaggatagcttacctcactgaggctaaggtggagaagctttgtgtgtggaacaacaagaccccccatgctattgctgccatcagcatggccaacgttactggtggtggaggatccgagaaggatgaactc

SEQ ID NO: 14 - protein, 115 aa, Artificial Sequence
  Cholera Toxin B Subunit Polypeptide Variant Polypeptide
TPQNITDLCAEYHNTQIHTLNDTIFSYTESLAGKREMAIITFKNGATFQVEVPGSQHIDSQKKAIERMKDTLRIAYLTEAKVEKLCVWNNKTPHAIAAISMANVTGGGGSEKDEL

SEQ ID NO: 15 - DNA, 393 bp, Artificial Sequence
  Cholera Toxin B Subunit Polypeptide Variant Polypeptide
atggctatcaagctcaagtttggagtgttcttcactgtgctccttagctctgcctatgcacatggcaccccacaaaacatcactgacttgtgtgctgagtaccacaacacccaaatccacaccctcaatgacaagatctttagctacaccgagagccttgctggcaagagggagatggctatcatcaccttcaagaatggtgctaccttccaagtggaggtgcctggaagccaacacattgatagccaaaagaaggccattgagaggatgaaggacacacttaggatagcttacctcactgaggctaaggtggagaagctttgtgtgtggaacaacaagaccccccatgctattgctgccatcagcatggccaactccgagaaggatgaactc

SEQ ID NO: 16 - protein, 131 aa, Artificial Sequence
  Cholera Toxin B Subunit Polypeptide Variant Polypeptide
MAIKLKFGVFFTVLLSSAYAHGTPQNITDLCAEYHNTQIHTLNDKIFSYTESLAGKREMAIITFKNGATFQVEVPGSQHIDSQKKAIERMKDTLRIAYLTEAKVEKLCVWNNKTPHAIAAISMANSEKDEL

SEQ ID NO: 17 - DNA, 78 bp, Oryza sativa
atggggaagcaaatggccgccctgtgtggctttctcctcgtggcgttgctctggctcacgcccgacgtcgcgcatggt

SEQ ID NO: 18 - protein, 26 aa, Oryza sativa
MGKQMAALCGFLLVALLWLTPDVAHG

SEQ ID NO: 19 - DNA, 81 bp, Nicotiana plumbaginifolia
atggctactcaacgaagggcaaaccctagctctctccatctaattactgtattctctctgctcgtcgctgtcgtctcaggt

SEQ ID NO: 20 - protein, 27 aa, Nicotiana plumbaginifolia
MATQRRANPSSLHLITVFSLLVAVVSG

SEQ ID NO: 21 - DNA, 78 bp, Malus domestica
atggcattgaagacacagttgttgtggtcattcgtggttgtgttcgttgtgtccttcagtacaacttcatgctcaggt

SEQ ID NO: 22 - protein, 26 aa, Malus domestica
MALKTQLLWSFVVVFVVSFSTTSCSG

SEQ ID NO: 23 - DNA, 72 bp, Hordeum vulgare
atggcgaacaaacacttgtccctctccctcttcctcgtcctccttggcctgtcggccagcttggcctcaggt

SEQ ID NO: 24 - protein, 24 aa, Hordeum vulgare
MANKHLSLSLFLVLLGLSASLASG

SEQ ID NO: 25 - protein, 109 aa, Artificial Sequence
  Cholera Toxin B Subunit Polypeptide Variant Polypeptide
TPQNITDLCAEYHNTQIHTLNDKIFCYTESLAGKREMAIITFKNGATFQVEVPGSQHIDSQKKAIERMKDTLRIAYLTEAKVEKLCVWNNKTPHAIAAISMCNSEKDEL

SEQ ID NO: 26 - protein, 135 aa, Artificial Sequence
  Cholera Toxin B Subunit Polypeptide Variant Polypeptide
MGKQMAALCGFLLVALLWLTPDVAHGTPQNITDLCAEYHNTQIHTLNDKIFSYTESLAGKREMAIITFKNGATFQVEVPGSQHIDSQKKAIERMKDTLRIAYLTEAKVEKLCVWNNKTPHAIAAISMANSEKDEL

SEQ ID NO: 27 - protein, 136 aa, Artificial Sequence
  Cholera Toxin B Subunit Polypeptide Variant Polypeptide
MATQRRANPSSLHLITVFSLLVAVVSGTPQNITDLCAEYHNTQIHTLNDKIFSYTESLAGKREMAIITFKNGATFQVEVPGSQHIDSQKKAIERMKDTLRIAYLTEAKVEKLCVWNNKTPHAIAAISMANSEKDEL

SEQ ID NO: 28 - protein, 135 aa, Artificial Sequence
  Cholera Toxin B Subunit Polypeptide Variant Polypeptide
MALKTQLLWSFVVVFVVSFSTTSCSGTPQNITDLCAEYHNTQIHTLNDKIFSYTESLAGKREMAIITFKNGATFQVEVPGSQHIDSQKKAIERMKDTLRIAYLTEAKVEKLCVWNNKTPHAIAAISMANSEKDEL

SEQ ID NO: 29 - protein, 133 aa, Artificial Sequence
  Cholera Toxin B Subunit Polypeptide Variant Polypeptide
MANKHLSLSLFLVLLGLSASLASGTPQNITDLCAEYHNTQIHTLNDKIFSYTESLAGKREMAIITFKNGATFQVEVPGSQHIDSQKKAIERMKDTLRIAYLTEAKVEKLCVWNNKTPHAIAAISMANSEKDEL

SEQ ID NO: 30 - protein, 6 aa, Artificial Sequence
  Endoplasmic Reticulum Retention Signal
SEKDEL

SEQ ID NO: 31 - protein, 4 aa, Artificial Sequence
  Endoplasmic Reticulum Retention Signal
KDEL